European Patent Application EP 4 778 944 A1, published July 22, 2026. Title: 可结合免疫检查点的多肽及其应用. Applicant: 重庆精准生物产业技术研究院有限公司. The sequence listing filed with the application follows.

SEQUENCE LISTING (35 sequences)

SEQ ID NO: 1 - protein, 236 aa, synthetic construct [sequence omitted]

SEQ ID NO: 2 - protein, 306 aa, synthetic construct
EEVLWHTSVPFAENMSLECVYPSMGILTQVEWFKIGTQQDSIAIFSPTHGMVIRKPYAERVYFLNSTMASNNMTLFFRNASEDDVGYYSCSLYTYPQGTWQKVIQVVQSDSFEAAVPSNSHIVSEPGKNVTLTCQPQMTWPVQAVRWEKIQPRQIDLLTYCNLVHGRNFTSKFPRQIVSNCSHGRWSVIVIPDVTVSDSGLYRCYLQASAGENETFVMRLTVAEGKTDNQYTLFVATRFWVLVVVGGVLACYSLLVTVAFIIFWVRSKRSRGGHSDYMNMTPRRPGPTRKHYQPYAPPRDFAAYRS

SEQ ID NO: 3 - protein, 254 aa, synthetic construct
MDYPTLLLALLHVYRALCEEVLWHTSVPFAENMSLECVYPSMGILTQVEWFKIGTQQDSIAIFSPTHGMVIRKPYAERVYFLNSTMASNNMTLFFRNASEDDVGYYSCSLYTYPQGTWQKVIQVVQSDSFEAAVPSNSHIVSEPGKNVTLTCQPQMTWPVQAVRWEKIQPRQIDLLTYCNLVHGRNFTSKFPRQIVSNCSHGRWSVIVIPDVTVSDSGLYRCYLQASAGENETFVMRLTVAEGKTDNQYTLFVA

SEQ ID NO: 4 - protein, 18 aa, synthetic construct
MDYPTLLLALLHVYRALC

SEQ ID NO: 5 - protein, 243 aa, synthetic construct
DIQLTQSPSSLSASVGDRVTITCKASQDVGTSVAWYQQKPGKAPKLLIYWTSTRHTGVPSRFSGSGSGTDFTFTISSLQPEDIATYYCQQYSLYRSFGQGTKVEIKGSTSGSGKPGSGEGSTKGEVQLVESGGGVVQPGRSLRLSCSASGFDFTTYWMSWVRQAPGKGLEWIGEIHPDSSTINYAPSLKDRFTISRDNAKNTLFLQMDSLRPEDTGVYFCASLYFGFPWFAYWGQGTPVTVSS

SEQ ID NO: 6 - protein, 468 aa, synthetic construct
DIQLTQSPSSLSASVGDRVTITCKASQDVGTSVAWYQQKPGKAPKLLIYWTSTRHTGVPSRFSGSGSGTDFTFTISSLQPEDIATYYCQQYSLYRSFGQGTKVEIKGSTSGSGKPGSGEGSTKGEVQLVESGGGVVQPGRSLRLSCSASGFDFTTYWMSWVRQAPGKGLEWIGEIHPDSSTINYAPSLKDRFTISRDNAKNTLFLQMDSLRPEDTGVYFCASLYFGFPWFAYWGQGTPVTVSSLETTTPAPRPPTPAPTIASQPLSLRPEACRPAAGGAVHTRGLDFACDIYIWAPLAGTCGVLLLSLVITLYCKRGRKKLLYIFKQPFMRPVQTTQEEDGCSCRFPEEEEGGCELRVKFSRSADAPAYKQGQNQLYNELNLGRREEYDVLDKRRGRDPEMGGKPRRKNPQEGLYNELQKDKMAEAYSEIGMKGERRRGKGHDGLYQGLSTATKDTYDALHMQALPPR

SEQ ID NO: 7 - protein, 816 aa, synthetic construct
DIQLTQSPSSLSASVGDRVTITCKASQDVGTSVAWYQQKPGKAPKLLIYWTSTRHTGVPSRFSGSGSGTDFTFTISSLQPEDIATYYCQQYSLYRSFGQGTKVEIKGSTSGSGKPGSGEGSTKGEVQLVESGGGVVQPGRSLRLSCSASGFDFTTYWMSWVRQAPGKGLEWIGEIHPDSSTINYAPSLKDRFTISRDNAKNTLFLQMDSLRPEDTGVYFCASLYFGFPWFAYWGQGTPVTVSSLETTTPAPRPPTPAPTIASQPLSLRPEACRPAAGGAVHTRGLDFACDIYIWAPLAGTCGVLLLSLVITLYCKRGRKKLLYIFKQPFMRPVQTTQEEDGCSCRFPEEEEGGCELRVKFSRSADAPAYKQGQNQLYNELNLGRREEYDVLDKRRGRDPEMGGKPRRKNPQEGLYNELQKDKMAEAYSEIGMKGERRRGKGHDGLYQGLSTATKDTYDALHMQALPPRVDGSGATNFSLLKQAGDVEENPGPMDYPTLLLALLHVYRALCEEVLWHTSVPFAENMSLECVYPSMGILTQVEWFKIGTQQDSIAIFSPTHGMVIRKPYAERVYFLNSTMASNNMTLFFRNASEDDVGYYSCSLYTYPQGTWQKVIQVVQSDSFEAAVPSNSHIVSEPGKNVTLTCQPQMTWPVQAVRWEKIQPRQIDLLTYCNLVHGRNFTSKFPRQIVSNCSHGRWSVIVIPDVTVSDSGLYRCYLQASAGENETFVMRLTVAEGKTDNQYTLFVATRFWVLVVVGGVLACYSLLVTVAFIIFWVRSKRSRGGHSDYMNMTPRRPGPTRKHYQPYAPPRDFAAYRS

SEQ ID NO: 8 - protein, 246 aa, synthetic construct
DIEMTQSPSSLSASVGDRVTITCRASQSISSHLNWYQQKSGKAPKLLIYAASSLQGGVPSRFSGSGSGTDFTLTISSLQPEDFATYYCQQSYSPPWTFGQGTKLELKRGSTSGSGKPGSGEGSTKGEVQLVQSGAEVKKPGSSVKVSCKASGGTFSSYAISWVRQAPGQGLEWMGGIIPIFGTANYAQKFQGRVTITADESTSTAYMELSSLRSEDTAVYYCARDTMIVANAFDIWGQGTTVTVSS

SEQ ID NO: 9 - protein, 471 aa, synthetic construct
DIEMTQSPSSLSASVGDRVTITCRASQSISSHLNWYQQKSGKAPKLLIYAASSLQGGVPSRFSGSGSGTDFTLTISSLQPEDFATYYCQQSYSPPWTFGQGTKLELKRGSTSGSGKPGSGEGSTKGEVQLVQSGAEVKKPGSSVKVSCKASGGTFSSYAISWVRQAPGQGLEWMGGIIPIFGTANYAQKFQGRVTITADESTSTAYMELSSLRSEDTAVYYCARDTMIVANAFDIWGQGTTVTVSSLETTTPAPRPPTPAPTIASQPLSLRPEACRPAAGGAVHTRGLDFACDIYIWAPLAGTCGVLLLSLVITLYCKRGRKKLLYIFKQPFMRPVQTTQEEDGCSCRFPEEEEGGCELRVKFSRSADAPAYKQGQNQLYNELNLGRREEYDVLDKRRGRDPEMGGKPRRKNPQEGLYNELQKDKMAEAYSEIGMKGERRRGKGHDGLYQGLSTATKDTYDALHMQALPPR

SEQ ID NO: 10 - protein, 819 aa, synthetic construct
DIEMTQSPSSLSASVGDRVTITCRASQSISSHLNWYQQKSGKAPKLLIYAASSLQGGVPSRFSGSGSGTDFTLTISSLQPEDFATYYCQQSYSPPWTFGQGTKLELKRGSTSGSGKPGSGEGSTKGEVQLVQSGAEVKKPGSSVKVSCKASGGTFSSYAISWVRQAPGQGLEWMGGIIPIFGTANYAQKFQGRVTITADESTSTAYMELSSLRSEDTAVYYCARDTMIVANAFDIWGQGTTVTVSSLETTTPAPRPPTPAPTIASQPLSLRPEACRPAAGGAVHTRGLDFACDIYIWAPLAGTCGVLLLSLVITLYCKRGRKKLLYIFKQPFMRPVQTTQEEDGCSCRFPEEEEGGCELRVKFSRSADAPAYKQGQNQLYNELNLGRREEYDVLDKRRGRDPEMGGKPRRKNPQEGLYNELQKDKMAEAYSEIGMKGERRRGKGHDGLYQGLSTATKDTYDALHMQALPPRVDGSGATNFSLLKQAGDVEENPGPMDYPTLLLALLHVYRALCEEVLWHTSVPFAENMSLECVYPSMGILTQVEWFKIGTQQDSIAIFSPTHGMVIRKPYAERVYFLNSTMASNNMTLFFRNASEDDVGYYSCSLYTYPQGTWQKVIQVVQSDSFEAAVPSNSHIVSEPGKNVTLTCQPQMTWPVQAVRWEKIQPRQIDLLTYCNLVHGRNFTSKFPRQIVSNCSHGRWSVIVIPDVTVSDSGLYRCYLQASAGENETFVMRLTVAEGKTDNQYTLFVATRFWVLVVVGGVLACYSLLVTVAFIIFWVRSKRSRGGHSDYMNMTPRRPGPTRKHYQPYAPPRDFAAYRS

SEQ ID NO: 11 - protein, 469 aa, synthetic construct
DIQMTQSPSSLSASVGDRVTITCRASQSISSYLNWYQQKPGKAPKLLIFAASSLQSGVPSRFSGSGSGTDFTLTISSLQPEDFATYYCQQSYSTPWTFGQGTKLDIKRGSTSGSGKPGSGEGSTKGEVQLVQSGPEVKKPGASVKVSCKASGYTFTDYYMNWVRQMHGKGLEWMGVINPYNGGTDYNQKFKGRVTITADKSTSTAYMELSSLRSEDTAVYYCARSVYDYPFDYWGQGTLVTVSSLETTTPAPRPPTPAPTIASQPLSLRPEACRPAAGGAVHTRGLDFACDIYIWAPLAGTCGVLLLSLVITLYCKRGRKKLLYIFKQPFMRPVQTTQEEDGCSCRFPEEEEGGCELRVKFSRSADAPAYKQGQNQLYNELNLGRREEYDVLDKRRGRDPEMGGKPRRKNPQEGLYNELQKDKMAEAYSEIGMKGERRRGKGHDGLYQGLSTATKDTYDALHMQALPPR

SEQ ID NO: 12 - protein, 817 aa, synthetic construct
DIQMTQSPSSLSASVGDRVTITCRASQSISSYLNWYQQKPGKAPKLLIFAASSLQSGVPSRFSGSGSGTDFTLTISSLQPEDFATYYCQQSYSTPWTFGQGTKLDIKRGSTSGSGKPGSGEGSTKGEVQLVQSGPEVKKPGASVKVSCKASGYTFTDYYMNWVRQMHGKGLEWMGVINPYNGGTDYNQKFKGRVTITADKSTSTAYMELSSLRSEDTAVYYCARSVYDYPFDYWGQGTLVTVSSLETTTPAPRPPTPAPTIASQPLSLRPEACRPAAGGAVHTRGLDFACDIYIWAPLAGTCGVLLLSLVITLYCKRGRKKLLYIFKQPFMRPVQTTQEEDGCSCRFPEEEEGGCELRVKFSRSADAPAYKQGQNQLYNELNLGRREEYDVLDKRRGRDPEMGGKPRRKNPQEGLYNELQKDKMAEAYSEIGMKGERRRGKGHDGLYQGLSTATKDTYDALHMQALPPRVDGSGATNFSLLKQAGDVEENPGPMDYPTLLLALLHVYRALCEEVLWHTSVPFAENMSLECVYPSMGILTQVEWFKIGTQQDSIAIFSPTHGMVIRKPYAERVYFLNSTMASNNMTLFFRNASEDDVGYYSCSLYTYPQGTWQKVIQVVQSDSFEAAVPSNSHIVSEPGKNVTLTCQPQMTWPVQAVRWEKIQPRQIDLLTYCNLVHGRNFTSKFPRQIVSNCSHGRWSVIVIPDVTVSDSGLYRCYLQASAGENETFVMRLTVAEGKTDNQYTLFVATRFWVLVVVGGVLACYSLLVTVAFIIFWVRSKRSRGGHSDYMNMTPRRPGPTRKHYQPYAPPRDFAAYRS

SEQ ID NO: 13 - protein, 45 aa, synthetic construct
TTTPAPRPPTPAPTIASQPLSLRPEACRPAAGGAVHTRGLDFACD

SEQ ID NO: 14 - protein, 21 aa, synthetic construct
IYIWAPLAGTCGVLLLSLVIT

SEQ ID NO: 15 - protein, 45 aa, synthetic construct
LYCKRGRKKLLYIFKQPFMRPVQTTQEEDGCSCRFPEEEEGGCEL

SEQ ID NO: 16 - protein, 112 aa, synthetic construct
RVKFSRSADAPAYKQGQNQLYNELNLGRREEYDVLDKRRGRDPEMGGKPRRKNPQEGLYNELQKDKMAEAYSEIGMKGERRRGKGHDGLYQGLSTATKDTYDALHMQALPPR

SEQ ID NO: 17 - protein, 27 aa, synthetic construct
FWVLVVVGGVLACYSLLVTVAFIIFWV

SEQ ID NO: 18 - protein, 41 aa, synthetic construct
RSKRSRGGHSDYMNMTPRRPGPTRKHYQPYAPPRDFAAYRS

SEQ ID NO: 19 - protein, 229 aa, synthetic construct
ESKYGPPCPPCPAPEFLGGPSVFLFPPKPKDTLMISRTPEVTCVVVDVSQEDPEVQFNWYVDGVEVHNAKTKPREEQFNSTYRVVSVLTVLHQDWLNGKEYKCKVSNKGLPSSIEKTISKAKGQPREPQVYTLPPSQEEMTKNQVSLTCLVKGFYPSDIAVEWESNGQPENNYKTTPPVLDSDGSFFLYSRLTVDKSRWQEGNVFSCSVMHEALHNHYTQKSLSLSLGK

SEQ ID NO: 20 - protein, 42 aa, synthetic construct
ALYLLRRDQRLPPDAHKPPGGGSFRTPIQEEQADAHSTLAKI

SEQ ID NO: 21 - protein, 36 aa, synthetic construct
APPRASALPAPPTGSALPDPQTASALPDPPAASALP

SEQ ID NO: 22 - protein, 45 aa, synthetic construct
KPTTTPAPRPPTPAPTIASQPLSLRPEARPAAGGAVHTRGLDFAD

SEQ ID NO: 23 - protein, 21 aa, synthetic construct
MALPVTALLLPLALLLHAARP

SEQ ID NO: 24 - protein, 22 aa, synthetic construct
GSGATNFSLLKQAGDVEENPGP

SEQ ID NO: 25 - DNA, 762 bp, synthetic construct
  source 1..762: mol_type = other DNA
atggattatcctactttacttttggctcttcttcatgtatacagagctctatgtgaagaggtgctttggcatacatcagttccctttgccgagaacatgtctctagaatgtgtgtatccatcaatgggcatcttaacacaggtggagtggttcaagatcgggacccagcaggattccatagccattttcagccctactcatggcatggtcataaggaagccctatgctgagagggtttactttttgaactcaacgatggcttccaataacatgactcttttctttcggaatgcctctgaagatgatgttggctactattcctgctctctttacacttacccacagggaacttggcagaaggtgatacaggtggttcagtcagatagttttgaggcagctgtgccatcaaatagccacattgtttcggaacctggaaagaatgtcacactcacttgtcagcctcagatgacgtggcctgtgcaggcagtgaggtgggaaaagatccagccccgtcagatcgacctcttaacttactgcaacttggtccatggcagaaatttcacctccaagttcccaagacaaatagtgagcaactgcagccacggaaggtggagcgtcatcgtcatccccgatgtcacagtctcagactcggggctttaccgctgctacttgcaggccagcgcaggagaaaacgaaaccttcgtgatgagattgactgtagccgagggtaaaaccgataaccaatataccctctttgtggct

SEQ ID NO: 26 - DNA, 972 bp, synthetic construct
  source 1..972: mol_type = other DNA
atggattatcctactttacttttggctcttcttcatgtatacagagctctatgtgaagaggtgctttggcatacatcagttccctttgccgagaacatgtctctagaatgtgtgtatccatcaatgggcatcttaacacaggtggagtggttcaagatcgggacccagcaggattccatagccattttcagccctactcatggcatggtcataaggaagccctatgctgagagggtttactttttgaactcaacgatggcttccaataacatgactcttttctttcggaatgcctctgaagatgatgttggctactattcctgctctctttacacttacccacagggaacttggcagaaggtgatacaggtggttcagtcagatagttttgaggcagctgtgccatcaaatagccacattgtttcggaacctggaaagaatgtcacactcacttgtcagcctcagatgacgtggcctgtgcaggcagtgaggtgggaaaagatccagccccgtcagatcgacctcttaacttactgcaacttggtccatggcagaaatttcacctccaagttcccaagacaaatagtgagcaactgcagccacggaaggtggagcgtcatcgtcatccccgatgtcacagtctcagactcggggctttaccgctgctacttgcaggccagcgcaggagaaaacgaaaccttcgtgatgagattgactgtagccgagggtaaaaccgataaccaatataccctctttgtggctactagattctgggtgctggtcgtggtgggtggcgtgctggcctgctacagcctgctggtgacagtggccttcatcatcttttgggtgaggagcaagcggagcagaggcggccacagcgactacatgaacatgactccccgccgccccgggcccacccgcaagcattaccagccctatgccccaccacgcgacttcgccgcctaccggagc

SEQ ID NO: 27 - DNA, 277 bp, synthetic construct
  source 1..277: mol_type = other DNA
atcccacagtgcatacgtgggctccaacaggtcctcttgtcgagccacagtgcatacgtgggctccaacaggtcctcttgtcgagccacagtgcatacgtgggctccaacaggtcctcttgtcgagccacagtgcatacgtgggctccaacaggtcctcttgtcgagccacagtgcatacgtgggctccaacaggtcctcttgtcgagatctggtaggcgtgtacggtgggaggtctatataagcagagctcgtttagtgaaccgtcagatcactag

SEQ ID NO: 28 - DNA, 545 bp, synthetic construct
  source 1..545: mol_type = other DNA
ggatctgcgatcgctccggtgcccgtcagtgggcagagcgcacatcgcccacagtccccgagaagttggggggaggggtcggcaattgaacgggtgcctagagaaggtggcgcggggtaaactgggaaagtgatgtcgtgtactggctccgcctttttcccgagggtgggggagaaccgtatataagtgcagtagtcgccgtgaacgttctttttcgcaacgggtttgccgccagaacacagctgaagcttcgaggggctcgcatctctccttcacgcgcccgccgccctacctgaggccgccatccacgccggttgagtcgcgttctgccgcctcccgcctgtggtgcctcctgaactgcgtccgccgtctaggtaagtttaaagctcaggtcgagaccgggcctttgtccggcgctcccttggagcctacctagactcagccggctctccacgctttgcctgaccctgcttgctcaactctacgtctttgtttcgttttctgttctgcgccgttacagatccaagctgtgaccggcgcctact

SEQ ID NO: 29 - DNA, 1404 bp, synthetic construct
  source 1..1404: mol_type = other DNA
gacatccagctgacccagtcccccagctccctgtccgcctctgtgggcgacagggtgaccatcacatgcaaggcctctcaggatgtgggcacaagcgtggcctggtatcagcagaagcccggcaaggcccctaagctgctgatctattggacctccacacggcacaccggcgtgcccagccggttcagcggctccggctctggcacagacttcaccttcaccatcagcagcctccagcccgaggacatcgccacctactattgtcagcagtacagcctgtatcggtcctttggccagggcacaaaggtggagatcaagggatccacttccggttcaggaaagcccgggagtggtgaaggtagcactaaaggcgaggtgcagctggtggagagcggaggaggagtggtgcagcctggccggtccctgagactgtcctgctctgccagcggcttcgactttaccacatactggatgtcctgggtgcggcaggcaccaggcaagggcctggagtggatcggcgagatccaccccgatagctccaccatcaactatgccccttccctgaaggacaggttcaccatctctcgcgataacgccaagaatacactgttcctccagatggactctctgaggcccgaggatacaggcgtgtacttctgtgccagcctgtatttcggctttccatggtttgcatactggggacagggcaccccagtgacagtgtctagcctcgagaccacgacgccagcgccgcgaccaccaacaccggcgcccaccatcgcgtcgcagcccctgtccctgcgcccagaggcgtgccggccagcggcggggggcgcagtgcacacgagggggctggacttcgcctgtgatatctacatctgggcgcccttggccgggacttgtggggtccttctcctgtcactggttatcaccctttactgcaaacggggcagaaagaaactcctgtatatattcaaacaaccatttatgagaccagtacaaactactcaagaggaagatggctgtagctgccgatttccagaagaagaagaaggaggatgtgaactgagagtgaagttcagcaggagcgcagacgcccccgcgtacaagcagggccagaaccagctctataacgagctcaatctaggacgaagagaggagtacgatgttttggacaagagacgtggccgggaccctgagatggggggaaagccgagaaggaagaaccctcaggaaggcctgtacaatgaactgcagaaagataagatggcggaggcctacagtgagattgggatgaaaggcgagcgccggaggggcaaggggcacgatggcctttaccagggtctcagtacagccaccaaggacacctacgacgcccttcacatgcaggccctgccccctcgc

SEQ ID NO: 30 - DNA, 2451 bp, synthetic construct
  source 1..2451: mol_type = other DNA
gacatccagctgacccagtcccccagctccctgtccgcctctgtgggcgacagggtgaccatcacatgcaaggcctctcaggatgtgggcacaagcgtggcctggtatcagcagaagcccggcaaggcccctaagctgctgatctattggacctccacacggcacaccggcgtgcccagccggttcagcggctccggctctggcacagacttcaccttcaccatcagcagcctccagcccgaggacatcgccacctactattgtcagcagtacagcctgtatcggtcctttggccagggcacaaaggtggagatcaagggatccacttccggttcaggaaagcccgggagtggtgaaggtagcactaaaggcgaggtgcagctggtggagagcggaggaggagtggtgcagcctggccggtccctgagactgtcctgctctgccagcggcttcgactttaccacatactggatgtcctgggtgcggcaggcaccaggcaagggcctggagtggatcggcgagatccaccccgatagctccaccatcaactatgccccttccctgaaggacaggttcaccatctctcgcgataacgccaagaatacactgttcctccagatggactctctgaggcccgaggatacaggcgtgtacttctgtgccagcctgtatttcggctttccatggtttgcatactggggacagggcaccccagtgacagtgtctagcctcgagaccacgacgccagcgccgcgaccaccaacaccggcgcccaccatcgcgtcgcagcccctgtccctgcgcccagaggcgtgccggccagcggcggggggcgcagtgcacacgagggggctggacttcgcctgtgatatctacatctgggcgcccttggccgggacttgtggggtccttctcctgtcactggttatcaccctttactgcaaacggggcagaaagaaactcctgtatatattcaaacaaccatttatgagaccagtacaaactactcaagaggaagatggctgtagctgccgatttccagaagaagaagaaggaggatgtgaactgagagtgaagttcagcaggagcgcagacgcccccgcgtacaagcagggccagaaccagctctataacgagctcaatctaggacgaagagaggagtacgatgttttggacaagagacgtggccgggaccctgagatggggggaaagccgagaaggaagaaccctcaggaaggcctgtacaatgaactgcagaaagataagatggcggaggcctacagtgagattgggatgaaaggcgagcgccggaggggcaaggggcacgatggcctttaccagggtctcagtacagccaccaaggacacctacgacgcccttcacatgcaggccctgccccctcgcgtcgacggaagcggagctactaacttcagcctgctgaagcaggctggagacgtggaggagaaccctggacctatggattatcctactttacttttggctcttcttcatgtatacagagctctatgtgaagaggtgctttggcatacatcagttccctttgccgagaacatgtctctagaatgtgtgtatccatcaatgggcatcttaacacaggtggagtggttcaagatcgggacccagcaggattccatagccattttcagccctactcatggcatggtcataaggaagccctatgctgagagggtttactttttgaactcaacgatggcttccaataacatgactcttttctttcggaatgcctctgaagatgatgttggctactattcctgctctctttacacttacccacagggaacttggcagaaggtgatacaggtggttcagtcagatagttttgaggcagctgtgccatcaaatagccacattgtttcggaacctggaaagaatgtcacactcacttgtcagcctcagatgacgtggcctgtgcaggcagtgaggtgggaaaagatccagccccgtcagatcgacctcttaacttactgcaacttggtccatggcagaaatttcacctccaagttcccaagacaaatagtgagcaactgcagccacggaaggtggagcgtcatcgtcatccccgatgtcacagtctcagactcggggctttaccgctgctacttgcaggccagcgcaggagaaaacgaaaccttcgtgatgagattgactgtagccgagggtaaaaccgataaccaatataccctctttgtggctactagattctgggtgctggtcgtggtgggtggcgtgctggcctgctacagcctgctggtgacagtggccttcatcatcttttgggtgaggagcaagcggagcagaggcggccacagcgactacatgaacatgactccccgccgccccgggcccacccgcaagcattaccagccctatgccccaccacgcgacttcgccgcctaccggagctaa

SEQ ID NO: 31 - DNA, 1416 bp, synthetic construct
  source 1..1416: mol_type = other DNA
gacatcgagatgacccagtctccatcctccctgtctgcatctgtaggagacagagtcaccatcacttgccgggcaagtcagagcatttccagccatttaaattggtatcagcagaaatcagggaaagcccctaagctcctgatctatgctgcgtccagtttgcaaggtggggtcccatcaaggttcagtggcagtggatctgggacagatttcactctcaccatcagcagtctgcaacctgaagattttgcaacttactactgtcaacagagttacagtcccccgtggacgttcggccaagggaccaagctggaactcaaacgtggcagcacaagcggaagcggcaaaccaggaagcggagaaggaagcaccaagggagaagtgcagctggtgcagtctggggctgaggtgaagaagcctgggtcctcggtgaaggtctcctgcaaggcttctggaggcaccttcagcagctatgctatcagctgggtgcgacaggcccctggacaagggcttgagtggatgggagggatcatccctatctttggtacagcaaactacgcacagaagttccagggcagagtcacgattaccgcggacgaatccacgagcacagcctacatggagctgagcagcctgagatctgaggacacggccgtgtattactgtgcgagagataccatgatagtagcaaatgcttttgatatctggggccaagggacaacggtcaccgtctcctcgctcgagaccacgacgccagcgccgcgaccaccaacaccggcgcccaccatcgcgtcgcagcccctgtccctgcgcccagaggcgtgccggccagcggcggggggcgcagtgcacacgagggggctggacttcgcctgtgatatctacatctgggcgcccttggccgggacttgtggggtccttctcctgtcactggttatcaccctttactgcaaacggggcagaaagaaactcctgtatatattcaaacaaccatttatgagaccagtacaaactactcaagaggaagatggctgtagctgccgatttccagaagaagaagaaggaggatgtgaactgagagtgaagttcagcaggagcgcagacgcccccgcgtacaagcagggccagaaccagctctataacgagctcaatctaggacgaagagaggagtacgatgttttggacaagagacgtggccgggaccctgagatggggggaaagccgagaaggaagaaccctcaggaaggcctgtacaatgaactgcagaaagataagatggcggaggcctacagtgagattgggatgaaaggcgagcgccggaggggcaaggggcacgatggcctttaccagggtctcagtacagccaccaaggacacctacgacgcccttcacatgcaggccctgccccctcgctaa

SEQ ID NO: 32 - DNA, 2460 bp, synthetic construct
  source 1..2460: mol_type = other DNA
gacatcgagatgacccagtctccatcctccctgtctgcatctgtaggagacagagtcaccatcacttgccgggcaagtcagagcatttccagccatttaaattggtatcagcagaaatcagggaaagcccctaagctcctgatctatgctgcgtccagtttgcaaggtggggtcccatcaaggttcagtggcagtggatctgggacagatttcactctcaccatcagcagtctgcaacctgaagattttgcaacttactactgtcaacagagttacagtcccccgtggacgttcggccaagggaccaagctggaactcaaacgtggcagcacaagcggaagcggcaaaccaggaagcggagaaggaagcaccaagggagaagtgcagctggtgcagtctggggctgaggtgaagaagcctgggtcctcggtgaaggtctcctgcaaggcttctggaggcaccttcagcagctatgctatcagctgggtgcgacaggcccctggacaagggcttgagtggatgggagggatcatccctatctttggtacagcaaactacgcacagaagttccagggcagagtcacgattaccgcggacgaatccacgagcacagcctacatggagctgagcagcctgagatctgaggacacggccgtgtattactgtgcgagagataccatgatagtagcaaatgcttttgatatctggggccaagggacaacggtcaccgtctcctcgctcgagaccacgacgccagcgccgcgaccaccaacaccggcgcccaccatcgcgtcgcagcccctgtccctgcgcccagaggcgtgccggccagcggcggggggcgcagtgcacacgagggggctggacttcgcctgtgatatctacatctgggcgcccttggccgggacttgtggggtccttctcctgtcactggttatcaccctttactgcaaacggggcagaaagaaactcctgtatatattcaaacaaccatttatgagaccagtacaaactactcaagaggaagatggctgtagctgccgatttccagaagaagaagaaggaggatgtgaactgagagtgaagttcagcaggagcgcagacgcccccgcgtacaagcagggccagaaccagctctataacgagctcaatctaggacgaagagaggagtacgatgttttggacaagagacgtggccgggaccctgagatggggggaaagccgagaaggaagaaccctcaggaaggcctgtacaatgaactgcagaaagataagatggcggaggcctacagtgagattgggatgaaaggcgagcgccggaggggcaaggggcacgatggcctttaccagggtctcagtacagccaccaaggacacctacgacgcccttcacatgcaggccctgccccctcgcgtcgacggaagcggagctactaacttcagcctgctgaagcaggctggagacgtggaggagaaccctggacctatggattatcctactttacttttggctcttcttcatgtatacagagctctatgtgaagaggtgctttggcatacatcagttccctttgccgagaacatgtctctagaatgtgtgtatccatcaatgggcatcttaacacaggtggagtggttcaagatcgggacccagcaggattccatagccattttcagccctactcatggcatggtcataaggaagccctatgctgagagggtttactttttgaactcaacgatggcttccaataacatgactcttttctttcggaatgcctctgaagatgatgttggctactattcctgctctctttacacttacccacagggaacttggcagaaggtgatacaggtggttcagtcagatagttttgaggcagctgtgccatcaaatagccacattgtttcggaacctggaaagaatgtcacactcacttgtcagcctcagatgacgtggcctgtgcaggcagtgaggtgggaaaagatccagccccgtcagatcgacctcttaacttactgcaacttggtccatggcagaaatttcacctccaagttcccaagacaaatagtgagcaactgcagccacggaaggtggagcgtcatcgtcatccccgatgtcacagtctcagactcggggctttaccgctgctacttgcaggccagcgcaggagaaaacgaaaccttcgtgatgagattgactgtagccgagggtaaaaccgataaccaatataccctctttgtggctactagattctgggtgctggtcgtggtgggtggcgtgctggcctgctacagcctgctggtgacagtggccttcatcatcttttgggtgaggagcaagcggagcagaggcggccacagcgactacatgaacatgactccccgccgccccgggcccacccgcaagcattaccagccctatgccccaccacgcgacttcgccgcctaccggagctaa

SEQ ID NO: 33 - DNA, 1410 bp, synthetic construct
  source 1..1410: mol_type = other DNA
gacatccagatgacccagtctccatcctccctgtctgcatctgtaggagacagagtcaccatcacttgccgggcaagtcagagcattagcagctatttaaattggtatcagcagaaaccagggaaagcccctaagctcctgatctttgctgcatccagtttgcaaagtggggtcccatcaaggttcagtggcagtggatctgggacagatttcactctcaccatcagcagtctgcaacctgaagattttgcaacttactactgtcaacagagttacagtaccccctggacgttcggccaagggaccaaactggatatcaaacgtggcagcacaagcggaagcggcaaaccaggaagcggagaaggaagcaccaagggagaggtgcagctggtgcagtccggaccagaggtgaagaagccaggagccagcgtgaaggtgtcctgtaaggcctctggctacaccttcacagattactatatgaactgggtgcggcagatgcacggcaagggactggagtggatgggcgtgatcaacccatacaatggcggcaccgattataatcagaagtttaagggcagagtgaccatcacagccgacaagtccacctctacagcctacatggagctgagctccctgaggagcgaggacacagccgtgtactattgtgcccgctccgtgtacgactatccctttgattattggggccagggcaccctggtcacagtctcctcactcgagaccacgacgccagcgccgcgaccaccaacaccggcgcccaccatcgcgtcgcagcccctgtccctgcgcccagaggcgtgccggccagcggcggggggcgcagtgcacacgagggggctggacttcgcctgtgatatctacatctgggcgcccttggccgggacttgtggggtccttctcctgtcactggttatcaccctttactgcaaacggggcagaaagaaactcctgtatatattcaaacaaccatttatgagaccagtacaaactactcaagaggaagatggctgtagctgccgatttccagaagaagaagaaggaggatgtgaactgagagtgaagttcagcaggagcgcagacgcccccgcgtacaagcagggccagaaccagctctataacgagctcaatctaggacgaagagaggagtacgatgttttggacaagagacgtggccgggaccctgagatggggggaaagccgagaaggaagaaccctcaggaaggcctgtacaatgaactgcagaaagataagatggcggaggcctacagtgagattgggatgaaaggcgagcgccggaggggcaaggggcacgatggcctttaccagggtctcagtacagccaccaaggacacctacgacgcccttcacatgcaggccctgccccctcgctaa

SEQ ID NO: 34 - DNA, 2454 bp, synthetic construct
  source 1..2454: mol_type = other DNA
gacatccagatgacccagtctccatcctccctgtctgcatctgtaggagacagagtcaccatcacttgccgggcaagtcagagcattagcagctatttaaattggtatcagcagaaaccagggaaagcccctaagctcctgatctttgctgcatccagtttgcaaagtggggtcccatcaaggttcagtggcagtggatctgggacagatttcactctcaccatcagcagtctgcaacctgaagattttgcaacttactactgtcaacagagttacagtaccccctggacgttcggccaagggaccaaactggatatcaaacgtggcagcacaagcggaagcggcaaaccaggaagcggagaaggaagcaccaagggagaggtgcagctggtgcagtccggaccagaggtgaagaagccaggagccagcgtgaaggtgtcctgtaaggcctctggctacaccttcacagattactatatgaactgggtgcggcagatgcacggcaagggactggagtggatgggcgtgatcaacccatacaatggcggcaccgattataatcagaagtttaagggcagagtgaccatcacagccgacaagtccacctctacagcctacatggagctgagctccctgaggagcgaggacacagccgtgtactattgtgcccgctccgtgtacgactatccctttgattattggggccagggcaccctggtcacagtctcctcactcgagaccacgacgccagcgccgcgaccaccaacaccggcgcccaccatcgcgtcgcagcccctgtccctgcgcccagaggcgtgccggccagcggcggggggcgcagtgcacacgagggggctggacttcgcctgtgatatctacatctgggcgcccttggccgggacttgtggggtccttctcctgtcactggttatcaccctttactgcaaacggggcagaaagaaactcctgtatatattcaaacaaccatttatgagaccagtacaaactactcaagaggaagatggctgtagctgccgatttccagaagaagaagaaggaggatgtgaactgagagtgaagttcagcaggagcgcagacgcccccgcgtacaagcagggccagaaccagctctataacgagctcaatctaggacgaagagaggagtacgatgttttggacaagagacgtggccgggaccctgagatggggggaaagccgagaaggaagaaccctcaggaaggcctgtacaatgaactgcagaaagataagatggcggaggcctacagtgagattgggatgaaaggcgagcgccggaggggcaaggggcacgatggcctttaccagggtctcagtacagccaccaaggacacctacgacgcccttcacatgcaggccctgccccctcgcgtcgacggaagcggagctactaacttcagcctgctgaagcaggctggagacgtggaggagaaccctggacctatggattatcctactttacttttggctcttcttcatgtatacagagctctatgtgaagaggtgctttggcatacatcagttccctttgccgagaacatgtctctagaatgtgtgtatccatcaatgggcatcttaacacaggtggagtggttcaagatcgggacccagcaggattccatagccattttcagccctactcatggcatggtcataaggaagccctatgctgagagggtttactttttgaactcaacgatggcttccaataacatgactcttttctttcggaatgcctctgaagatgatgttggctactattcctgctctctttacacttacccacagggaacttggcagaaggtgatacaggtggttcagtcagatagttttgaggcagctgtgccatcaaatagccacattgtttcggaacctggaaagaatgtcacactcacttgtcagcctcagatgacgtggcctgtgcaggcagtgaggtgggaaaagatccagccccgtcagatcgacctcttaacttactgcaacttggtccatggcagaaatttcacctccaagttcccaagacaaatagtgagcaactgcagccacggaaggtggagcgtcatcgtcatccccgatgtcacagtctcagactcggggctttaccgctgctacttgcaggccagcgcaggagaaaacgaaaccttcgtgatgagattgactgtagccgagggtaaaaccgataaccaatataccctctttgtggctactagattctgggtgctggtcgtggtgggtggcgtgctggcctgctacagcctgctggtgacagtggccttcatcatcttttgggtgaggagcaagcggagcagaggcggccacagcgactacatgaacatgactccccgccgccccgggcccacccgcaagcattaccagccctatgccccaccacgcgacttcgccgcctaccggagctaa

SEQ ID NO: 35 - protein, 244 aa, synthetic construct
DIQMTQSPSSLSASVGDRVTITCRASQSISSYLNWYQQKPGKAPKLLIFAASSLQSGVPSRFSGSGSGTDFTLTISSLQPEDFATYYCQQSYSTPWTFGQGTKLDIKRGSTSGSGKPGSGEGSTKGEVQLVQSGPEVKKPGASVKVSCKASGYTFTDYYMNWVRQMHGKGLEWMGVINPYNGGTDYNQKFKGRVTITADKSTSTAYMELSSLRSEDTAVYYCARSVYDYPFDYWGQGTLVTVSS